European Patent Application EP 4 790 139 A1, published August 12, 2026. Title: ポリペプチドの会合体形成抑制方法. Applicant: NATIONAL UNIVERSITY CORPORATION KUMAMOTO UNIVERSITY. Application WO. The sequence listing filed with the application follows.

SEQUENCE LISTING (52 sequences)

SEQ ID NO: 1 - protein, 11 aa, Artificial Sequence
  VARIANT 1..3: note = any natural amino acid
  VARIANT 5: note = any natural amino acid
  VARIANT 8: note = any natural amino acid
  VARIANT 10..11: note = any natural amino acid
XXXGXGQXWXX

SEQ ID NO: 2 - protein, 13 aa, Artificial Sequence
  VARIANT 2..4: note = any natural amino acid
  VARIANT 7..12: note = any natural amino acid
AXXXSGXXXXXXT

SEQ ID NO: 3 - protein, 10 aa, Artificial Sequence
TAGAGQSWYG

SEQ ID NO: 4 - protein, 13 aa, Artificial Sequence
AAGGSGSGADGAT

SEQ ID NO: 5 - protein, 24 aa, Artificial Sequence
  VARIANT 1: note = any natural amino acid
  VARIANT 3..12: note = any natural amino acid
  VARIANT 14..16: note = any natural amino acid
  VARIANT 18: note = any natural amino acid
  VARIANT 21: note = any natural amino acid
  VARIANT 23..24: note = any natural amino acid
XPXXXXXXXXXXGXXXGXGQXWXX

SEQ ID NO: 6 - protein, 22 aa, Artificial Sequence
  VARIANT 1..3: note = any natural amino acid
  VARIANT 10..15: note = any natural amino acid
  VARIANT 5..7: note = any natural amino acid
  VARIANT 17..22: note = any natural amino acid
XXXAXXXSGXXXXXXTXXXXXX

SEQ ID NO: 7 - protein, 24 aa, Artificial Sequence
XPXXXXXXXXXXGATAGAGQSWYG

SEQ ID NO: 8 - protein, 22 aa, Artificial Sequence
  VARIANT 1..3: note = any natural amino acid
  VARIANT 17..22: note = any natural amino acid
XXXAAGGSGSGADGATXXXXXX

SEQ ID NO: 9 - protein, 24 aa, Artificial Sequence
GPEEQYSAYATTGATAGAGQSWYG

SEQ ID NO: 10 - protein, 22 aa, Artificial Sequence
PGAAAGGSGSGADGATYTTTPG

SEQ ID NO: 11 - protein, 255 aa, Artificial Sequence
MEVQLVESGGGLVQPGGSLRLSCAASGFNIKDTYIHWVRQAPGKGLEWVARIYPTNGYTRYADSVKGRFTISADTSKNTAYLQMNSLRAEDTAVYYCSRWGGDGFYAMDYWGQGTLVTVSSGGGGSGGGGSGGGGSDIQMTQSPSSLSASVGDRVTITCRASQDVNTAVAWYQQKPGKAPKLLIYSASFLYSGVPSRFSGSRSGTDFTLTISSLQPEDFATYYCQQHYTTPPTFGQGTKVEIKSAAALEHHHHHH

SEQ ID NO: 12 - DNA, 768 bp, Artificial Sequence
  source 1..768: mol_type = other DNA
atggaagtgcagctggttgaaagcggtggcggtctggtgcaaccgggcggtagcctgcgtctgagctgcgcggcgagcggttttaacatcaaagacacctacattcactgggttcgtcaagcgccgggcaagggtctggagtgggttgcgcgtatctatccgaccaacggctacacccgttatgcggacagcgtgaaaggtcgttttaccattagcgcggataccagcaagaacaccgcgtacctgcagatgaacagcctgcgtgcggaagacaccgcggtttactattgcagccgttggggcggtgacggcttctacgcgatggattattggggccaaggcaccctggtgaccgttagcagcggcggtggaggtagtggtggtggaggttccggtggtggcggtagcgatatccagatgacccagagcccgagcagcctgagcgcgagcgtgggtgaccgtgttaccattacctgccgtgcgagccaagatgtgaacaccgcggttgcgtggtatcagcaaaagccgggcaaagcgccgaagctgctgatctacagcgcgagcttcctgtatagcggtgtgccgagccgttttagcggcagccgtagcggcaccgacttcaccctgaccattagcagcctgcagccggaggattttgcgacctactattgccagcaacactataccaccccgccgacctttggtcaaggcaccaaagttgaaatcaagagcgcggccgcactcgagcaccaccaccaccaccactga

SEQ ID NO: 13 - DNA, 570 bp, Artificial Sequence
  source 1..570: mol_type = other DNA
atgaaagcaatagataaaatgacggataatccaccacaagaaggcttaagtgggaggaaaataatatatgacgaagatggcaaaccttgccgatcatgtaacaccctacttgactttcagtacgtgaccgggaagatatctaatggcctgaagaacctctcatctaacggtaaactagcaggtacgggggctctcactggcgaagcttcagagttgatgcctggctcaagaacatacaggaaggttgaccctcctgacgtagagcaactaggtagatcttcatggacgctgttacactctgtagctgccagctatcctgctcaacctacagaccaacagaagggtgaaatgaaacagttcttgaatatcttctcacatatttatccttgcaactggtgtgctaaagactttgaaaaatatatcagagaaaatgcaccacaagttgagtcaagagaagaacttgggaggtggatgtgtgaagcccacaataaagtcaataagaaattgaggaagcccaaatttgactgtaatttctgggaaaaaagatggaaggacggctgggacgaataa

SEQ ID NO: 14 - protein, 189 aa, Artificial Sequence
MKAIDKMTDNPPQEGLSGRKIIYDEDGKPCRSCNTLLDFQYVTGKISNGLKNLSSNGKLAGTGALTGEASELMPGSRTYRKVDPPDVEQLGRSSWTLLHSVAASYPAQPTDQQKGEMKQFLNIFSHIYPCNWCAKDFEKYIRENAPQVESREELGRWMCEAHNKVNKKLRKPKFDCNFWEKRWKDGWDE

SEQ ID NO: 15 - DNA, 43 bp, Artificial Sequence
  source 1..43: mol_type = other DNA
cgagatctcgatctcctttgttcgacttaagcattattcgtcc

SEQ ID NO: 16 - DNA, 37 bp, Artificial Sequence
  source 1..37: mol_type = other DNA
ggccacgatgcgtccctgacctcctatgcactcctgc

SEQ ID NO: 17 - DNA, 40 bp, Artificial Sequence
  source 1..40: mol_type = other DNA
gaggatcgagatctcgatccgcgaaattaatacgactcac

SEQ ID NO: 18 - DNA, 28 bp, Artificial Sequence
  source 1..28: mol_type = other DNA
ggacgcatcgtggccggcatcaccggcc

SEQ ID NO: 19 - DNA, 60 bp, Artificial Sequence
  source 1..60: mol_type = other DNA
catggtatatctccttcttaaagttaaacaaaattatttctagaggggaattgttatccg

SEQ ID NO: 20 - DNA, 25 bp, Artificial Sequence
  source 1..25: mol_type = other DNA
gcggccgcactcgagcaccaccacc

SEQ ID NO: 21 - DNA, 789 bp, Artificial Sequence
  source 1..789: mol_type = other DNA
ctttaagaaggagatataccatggaagtgcagctggttgaaagcggtggcggtctggtgcaaccgggcggtagcctgcgtctgagctgcgcggcgagcggttttaacatcaaagacacctacattcactgggttcgtcaagcgccgggcaagggtctggagtgggttgcgcgtatctatccgaccaacggctacacccgttatgcggacagcgtgaaaggtcgttttaccattagcgcggataccagcaagaacaccgcgtacctgcagatgaacagcctgcgtgcggaagacaccgcggtttactattgcagccgttggggcggtgacggcttctacgcgatggattattggggccaaggcaccctggtgaccgttggcccggaagaacagtatagcgcgtatgcgaccaccggcgcgaccgcgggcgcgggccagagctggtatggcgaaatccagatgacccagagcccgagcagcctgagcgcgagcgtgggtgaccgtgttaccattacctgccgtgcgagccaagatgtgaacaccgcggttgcgtggtatcagcaaaagccgggcaaagcgccgaagctgctgatctacagcgcgagcttcctgtatagcggtgtgccgagccgttttagcggcagccgtagcggcaccgacttcaccctgaccattagcagcctgcagccggaggattttgcgacctactattgccagcaacactataccaccccgccgacctttggtcaaggcaccaaagttgaaatcaagagcgcggccgcactcgagc

SEQ ID NO: 22 - protein, 262 aa, Artificial Sequence
MEVQLVESGGGLVQPGGSLRLSCAASGFNIKDTYIHWVRQAPGKGLEWVARIYPTNGYTRYADSVKGRFTISADTSKNTAYLQMNSLRAEDTAVYYCSRWGGDGFYAMDYWGQGTLVTVGPEEQYSAYATTGATAGAGQSWYGEIQMTQSPSSLSASVGDRVTITCRASQDVNTAVAWYQQKPGKAPKLLIYSASFLYSGVPSRFSGSRSGTDFTLTISSLQPEDFATYYCQQHYTTPPTFGQGTKVEIKSAAALEHHHHHH

SEQ ID NO: 23 - DNA, 753 bp, Artificial Sequence
  source 1..753: mol_type = other DNA
atggaagtgcagctggttgaaagcggtggcggtctggtgcaaccgggcggtagcctgcgtctgagctgcgcggcgagcggttttaacatcaaagacacctacattcactgggttcgtcaagcgccgggcaagggtctggagtgggttgcgcgtatctatccgaccaacggctacacccgttatgcggacagcgtgaaaggtcgttttaccattagcgcggataccagcaagaacaccgcgtacctgcagatgaacagcctgcgtgcggaagacaccgcggtttactattgcagccgttggggcggtgacggcttctacgcgatggattattggggccaaggcaccctggtgaccgttggcccggaagaacagtatagcgcgtatgcgaccaccggcgcgaccgcgggcgcgggccagagctggtatggcgaaatccagatgacccagagcccgagcagcctgagcgcgagcgtgggtgaccgtgttaccattacctgccgtgcgagccaagatgtgaacaccgcggttgcgtggtatcagcaaaagccgggcaaagcgccgaagctgctgatctacagcgcgagcttcctgtatagcggtgtgccgagccgttttagcggcagccgtagcggcaccgacttcaccctgaccattagcagcctgcagccggaggattttgcgacctactattgccagcaacactataccaccccgccgacctttggtcaaggcaccaaagttgaaatcaagagc

SEQ ID NO: 24 - DNA, 47 bp, Artificial Sequence
  source 1..47: mol_type = other DNA
caggggccccatatggcccaggtgaaactgcagcagtcaggacctag

SEQ ID NO: 25 - DNA, 46 bp, Artificial Sequence
  source 1..46: mol_type = other DNA
ctcgagtgcggccgctatttccaactttgtcccccctccgaacgtg

SEQ ID NO: 26 - DNA, 32 bp, Artificial Sequence
  source 1..32: mol_type = other DNA
catatggggcccctggaacagaacttccagcg

SEQ ID NO: 27 - protein, 257 aa, Artificial Sequence
GPHMAQVKLQQSGPSLVKPSQTLSLTCSVTGDSITSGYWNWIRKFPGNKFEYLGYISYSGRTYYNPSLKSRISITRDTSKNQYYLQLNSVTTEDTATYYCSRPYYRYDYAIDYWGQGTTVTVSSGGGGSGGGGSGGGGSDIELTQSPAIMSASLGEQVTMTCTASSSVSSSYLHWYQQKPGSSPKLWIYSTSNLASGVPARFSSSGSGTSYSLTISRMEAEDAATYYCQQSWKAPYTFGGGTKLEIAAALEHHHHHH

SEQ ID NO: 28 - DNA, 726 bp, Artificial Sequence
  source 1..726: mol_type = other DNA
gcccaggtgaaactgcagcagtcaggacctagcctcgtgaaaccttctcagactctgtccctcacctgttctgtcactggcgactccatcaccagtggttactggaactggatccggaaattcccagggaataaatttgagtacttgggttacataagctacagtggtcgcacttactacaatccatctctcaaaagtcgaatctccatcactcgagacacatccaagaaccagtactacctgcagttgaattctgtgactactgaggacacagccacatattactgttcaagaccctactataggtacgactatgctatagactactggggccaagggaccacggtcaccgtctcctcaggtggaggcggttcaggcggaggtggctctggcggtggcggatcggacatcgagctcactcagtctccagcaatcatgtctgcatctctaggggaacaggtcaccatgacctgcactgccagctcaagtgtaagttccagttacttgcactggtaccagcagaagccaggatcctcccccaaactctggatttatagcacatccaacctggcttctggagtcccagctcgcttcagtagcagtggatctgggacctcttactctctcacaatcagccgaatggaggctgaagatgctgccacctattactgccagcaaagttggaaggccccgtacacgttcggaggggggacaaagttggaaata

SEQ ID NO: 29 - DNA, 39 bp, Artificial Sequence
  source 1..39: mol_type = other DNA
gacggtgaccgtggtcccttggccccagtagtctatagc

SEQ ID NO: 30 - DNA, 44 bp, Artificial Sequence
  source 1..44: mol_type = other DNA
atcgagctcactcagtctccagcaatcatgtctgcatctctagg

SEQ ID NO: 31 - DNA, 46 bp, Artificial Sequence
  source 1..46: mol_type = other DNA
gaccacggtcaccgtcggcccggaagaacagtatagcgcgtatgcg

SEQ ID NO: 32 - DNA, 46 bp, Artificial Sequence
  source 1..46: mol_type = other DNA
gagactgagtgagctcgatttcgccataccagctctggcccgcgcc

SEQ ID NO: 33 - protein, 264 aa, Artificial Sequence
GPHMAQVKLQQSGPSLVKPSQTLSLTCSVTGDSITSGYWNWIRKFPGNKFEYLGYISYSGRTYYNPSLKSRISITRDTSKNQYYLQLNSVTTEDTATYYCSRPYYRYDYAIDYWGQGTTVTVGPEEQYSAYATTGATAGAGQSWYGEIELTQSPAIMSASLGEQVTMTCTASSSVSSSYLHWYQQKPGSSPKLWIYSTSNLASGVPARFSSSGSGTSYSLTISRMEAEDAATYYCQQSWKAPYTFGGGTKLEIAAALEHHHHHH

SEQ ID NO: 34 - DNA, 768 bp, Artificial Sequence
  source 1..768: mol_type = other DNA
ctttaagaaggagatataccatggatatccagatgacccagagcccgagcagcctgagcgcgagcgtgggtgaccgtgttaccattacctgccgtgcgagccaagatgtgaacaccgcggttgcgtggtatcagcaaaagccgggcaaagcgccgaagctgctgatctacagcgcgagcttcctgtatagcggtgtgccgagccgttttagcggcagccgtagcggcaccgacttcaccctgaccattagcagcctgcagccggaggattttgcgacctactattgccagcaacactataccaccccgccgacctttggtcaaggcaccaaagttgaaatcggtagcggtggcggaggtagcggtggtggcggtagtggtggtggaggttccgaagtgcagctggttgaaagcggtggcggtctggtgcaaccgggcggtagcctgcgtctgagctgcgcggcgagcggttttaacatcaaagacacctacattcactgggttcgtcaagcgccgggcaagggtctggagtgggttgcgcgtatctatccgaccaacggctacacccgttatgcggacagcgtgaaaggtcgttttaccattagcgcggataccagcaagaacaccgcgtacctgcagatgaacagcctgcgtgcggaagacaccgcggtttactattgcagccgttggggcggtgacggcttctacgcgatggattattggggccaaggcaccctggtgaccgttagcagcgcggccgcactcgagc

SEQ ID NO: 35 - DNA, 50 bp, Artificial Sequence
  source 1..50: mol_type = other DNA
ctttaagaaggagatataccatggatatccagatgacccagagcccgagc

SEQ ID NO: 36 - DNA, 45 bp, Artificial Sequence
  source 1..45: mol_type = other DNA
gctcgagtgcggccgcgctgctaacggtcaccagggtgccttggc

SEQ ID NO: 37 - protein, 255 aa, Artificial Sequence
MDIQMTQSPSSLSASVGDRVTITCRASQDVNTAVAWYQQKPGKAPKLLIYSASFLYSGVPSRFSGSRSGTDFTLTISSLQPEDFATYYCQQHYTTPPTFGQGTKVEIGSGGGGSGGGGSGGGGSEVQLVESGGGLVQPGGSLRLSCAASGFNIKDTYIHWVRQAPGKGLEWVARIYPTNGYTRYADSVKGRFTISADTSKNTAYLQMNSLRAEDTAVYYCSRWGGDGFYAMDYWGQGTLVTVSSAAALEHHHHHH

SEQ ID NO: 38 - DNA, 885 bp, Artificial Sequence
  source 1..885: mol_type = other DNA
ctttaagaaggagatataccatggacattcagatgacccaaagtccatcaagtctttccgcgtcagtcggcgaccgcgttacaattacttgtcgcgcatcgcaggacgtaaacacggccgtggcttggtaccaacagaagcccggtaaagccccaaagctgttgatctactctgcctcattcttatatagcggagtcccttctcgcttctctggctcgcgcagtggtacagactttactttgacgatctctagcctgcaacctgaagacttcgcgacatactactgtcaacagcattatactaccccacctacttttggtcagggaacgaaggtagaaatcgtagaaatcggtcccgcagctgctgccactagcacttatacgtacgctactgccactgcgacaactggaaccacgtcctacacggctaacacaaccggacgcccgggtgctgccgcaggtggttccggaagcggtgctgacggcgcaacttacacgaccacgccaggtcaagtccagctggtggagtccggtggaggcctggtgcagcctggcggctccttacgtctgtcttgtgctgcctccggtttcaacattaaggacacctacatccactgggttcgccaggcacccggtaaaggtcttgagtgggtggcacgtatttacccaactaatggctacactcgctacgctgacagcgtaaaagggcgctttactatctccgcagataccagcaaaaacacggcatacctgcaaatgaattcacttcgtgctgaagacacggcagtgtattactgctcacgctggggcggagacggattctacgcaatggactattgggggcagggcacgttggtgacagttagttcagcggccgcactcgagc

SEQ ID NO: 39 - protein, 294 aa, Artificial Sequence
MDIQMTQSPSSLSASVGDRVTITCRASQDVNTAVAWYQQKPGKAPKLLIYSASFLYSGVPSRFSGSRSGTDFTLTISSLQPEDFATYYCQQHYTTPPTFGQGTKVEIVEIGPAAAATSTYTYATATATTGTTSYTANTTGRPGAAAGGSGSGADGATYTTTPGQVQLVESGGGLVQPGGSLRLSCAASGFNIKDTYIHWVRQAPGKGLEWVARIYPTNGYTRYADSVKGRFTISADTSKNTAYLQMNSLRAEDTAVYYCSRWGGDGFYAMDYWGQGTLVTVSSAAALEHHHHHH

SEQ ID NO: 40 - DNA, 838 bp, Artificial Sequence
  source 1..838: mol_type = other DNA
ctttaagaaggagatataccatgggcagcagccatcatcatcatcatcactccagctcgctggaagttctgttccaggggccccatatggacatcgagctcactcagtctccagcaatcatgtctgcatctctaggggaacaggtcaccatgacctgcactgccagctcaagtgtaagttccagttacttgcactggtaccagcagaagccaggatcctcccccaaactctggatttatagcacatccaacctggcttctggagtcccagctcgcttcagtagcagtggatctgggacctcttactctctcacaatcagccgaatggaggctgaagatgctgccacctattactgccagcaaagttggaaggccccgtacacgttcggaggggggacaaagttggaaataggcagcggtggaggcggttcaggcggaggtggctctggcggtggcggatcgcaggtgaaactgcagcagtcaggacctagcctcgtgaaaccttctcagactctgtccctcacctgttctgtcactggcgactccatcaccagtggttactggaactggatccggaaattcccagggaataaatttgagtacttgggttacataagctacagtggtcgcacttactacaatccatctctcaaaagtcgaatctccatcactcgagacacatccaagaaccagtactacctgcagttgaattctgtgactactgaggacacagccacatattactgttcaagaccctactataggtacgactatgctatagactactggggccaagggaccacggtcaccgtctcctcataatgcggccgcactcgagc

SEQ ID NO: 41 - protein, 266 aa, Artificial Sequence
MGSSHHHHHHSSSLEVLFQGPHMDIELTQSPAIMSASLGEQVTMTCTASSSVSSSYLHWYQQKPGSSPKLWIYSTSNLASGVPARFSSSGSGTSYSLTISRMEAEDAATYYCQQSWKAPYTFGGGTKLEIGSGGGGSGGGGSGGGGSQVKLQQSGPSLVKPSQTLSLTCSVTGDSITSGYWNWIRKFPGNKFEYLGYISYSGRTYYNPSLKSRISITRDTSKNQYYLQLNSVTTEDTATYYCSRPYYRYDYAIDYWGQGTTVTVSS

SEQ ID NO: 42 - DNA, 946 bp, Artificial Sequence
  source 1..946: mol_type = other DNA
ctttaagaaggagatataccatgggcagccatcaccatcaccatcattcatcatcattagaagtcttagagttcggtccacatatggctgatatcgaattaactcagtctcccgcaatcatgtcggccagcttaggtgagcaggtaacaatgacttgtaccgcttcttcgagtgtatcgtcgagttacctgcactggtaccaacaaaaaccaggttcttctcccaaactgtggatttattcaacctcaaaccttgcatctggcgtccccgctcgcttctcatcgtctggatcgggtacaagttattctcttacgatttctcgcatggaggcagaagacgcagctacctattattgccagcaatcttggaaggcgccttacacgttcggcggagggacaaaattggaaattggacccgccgctgcagcgacctcgacatacacctacgcgactgccacagcgacaacaggaacaactagctacacggcaaatacaacaggccgcccgggagctgccgccgggggttcaggaagtggagccgacggtgcaacttataccaccacacctgggcaagtcaaacttcaacagagcggcccgtcattggtgaaaccctcgcagacccttagtttgacctgttcggtgaccggagacagcattacatctggctattggaactggattcgcaaatttcctggtaacaaattcgagtatcttggctatattagctattctggacgtacctactacaatccatcccttaaatctcgtatttccatcacccgcgacacttcaaaaaatcagtattatttgcaactgaattcggtcactacagaagacacggctacctactattgttcacgtccgtattatcgctatgactatgctattgattactgggggcaggggacgaccgttactgtgtcatcttaatgcggccgcactcgagc

SEQ ID NO: 43 - protein, 302 aa, Artificial Sequence
MGSHHHHHHSSSLEVLEFGPHMADIELTQSPAIMSASLGEQVTMTCTASSSVSSSYLHWYQQKPGSSPKLWIYSTSNLASGVPARFSSSGSGTSYSLTISRMEAEDAATYYCQQSWKAPYTFGGGTKLEIGPAAAATSTYTYATATATTGTTSYTANTTGRPGAAAGGSGSGADGATYTTTPGQVKLQQSGPSLVKPSQTLSLTCSVTGDSITSGYWNWIRKFPGNKFEYLGYISYSGRTYYNPSLKSRISITRDTSKNQYYLQLNSVTTEDTATYYCSRPYYRYDYAIDYWGQGTTVTVSS

SEQ ID NO: 44 - DNA, 874 bp, Artificial Sequence
  source 1..874: mol_type = other DNA
ctttaagaaggagatataccatgggttcccatcatcaccaccaccactcatcctcacttgaggtactggagtttcaggggccacatatgggttccaccgccggtgcaggacagtcctggtatggagagatccaaatgacgcagtcgccctcgtcgctttcggcctccgtgggagaccgcgtcacaattacgtgccgcgcgtcgcaagatgtaaacaccgccgttgcgtggtatcaacagaaaccaggtaaagcaccgaaacttcttatttactccgccagttttttatattcgggtgtcccatcccgtttttccggctcgcgctctggcacagacttcactctgacaatttcctccctgcagccggaagatttcgcgacttattattgccagcaacattatactaccccacctacgtttgggcaaggtactaaggtagaaatcggttcaggcggcggtggctcaggtggagggggttccggtgggggtggatcggaggtccagcttgtagaaagcggtggaggtttagtacaaccaggggggtctcttcgtctttcttgcgcggcgtcgggattcaatatcaaggatacttacattcactgggtacgccaagcgcccgggaaggggcttgagtgggtggcacgtatctaccccactaacggatatacccgttatgccgattctgtcaaagggcgctttaccatcagcgcagatacgagcaaaaatacggcgtaccttcaaatgaattcgctgcgtgctgaagacacagcagtttattactgttcccgctggggcggcgacggcttctacgctatggattactggggccaaggcacattggtcactgtgtcatcctaatgcggccgcactcgagc

SEQ ID NO: 45 - protein, 278 aa, Artificial Sequence
MGSHHHHHHSSSLEVLEFQGPHMGSTAGAGQSWYGEIQMTQSPSSLSASVGDRVTITCRASQDVNTAVAWYQQKPGKAPKLLIYSASFLYSGVPSRFSGSRSGTDFTLTISSLQPEDFATYYCQQHYTTPPTFGQGTKVEIGSGGGGSGGGGSGGGGSEVQLVESGGGLVQPGGSLRLSCAASGFNIKDTYIHWVRQAPGKGLEWVARIYPTNGYTRYADSVKGRFTISADTSKNTAYLQMNSLRAEDTAVYYCSRWGGDGFYAMDYWGQGTLVTVSS

SEQ ID NO: 46 - protein, 15 aa, Artificial Sequence
GGGGSGGGGSGGGGS

SEQ ID NO: 47 - protein, 24 aa, Artificial Sequence
GGGGSGGGGSGGGSTAGAGQSWYG

SEQ ID NO: 48 - protein, 5 aa, Artificial Sequence
GGGGS

SEQ ID NO: 49 - protein, 4 aa, Artificial Sequence
GGGS

SEQ ID NO: 50 - protein, 14 aa, Artificial Sequence
GGGGSGGGGSGGGS

SEQ ID NO: 51 - protein, 250 aa, Artificial Sequence
EVQLVESGGGLVQPGGSLRLSCAASGFNIKDTYIHWVRQAPGKGLEWVARIYPTNGYTRYADSVKGRFTISADTSKNTAYLQMNSLRAEDTAVYYCSRWGGDGFYAMDYWGQGTLVTVGGGGSGGGGSGGGSTAGAGQSWYGEIQMTQSPSSLSASVGDRVTITCRASQDVNTAVAWYQQKPGKAPKLLIYSASFLYSGVPSRFSGSRSGTDFTLTISSLQPEDFATYYCQQHYTTPPTFGQGTKVEIKS

SEQ ID NO: 52 - DNA, 789 bp, Artificial Sequence
  source 1..789: mol_type = other DNA
ctttaagaaggagatataccatggaagtgcagctggttgaaagcggtggcggtctggtgcaaccgggcggtagcctgcgtctgagctgcgcggcgagcggttttaacatcaaagacacctacattcactgggttcgtcaagcgccgggcaagggtctggagtgggttgcgcgtatctatccgaccaacggctacacccgttatgcggacagcgtgaaaggtcgttttaccattagcgcggataccagcaagaacaccgcgtacctgcagatgaacagcctgcgtgcggaagacaccgcggtttactattgcagccgttggggcggtgacggcttctacgcgatggattattggggccaaggcaccctggtgaccgttgggggagggggttcgggtggggggggttcggggggaggcagcactgcaggagctggtcaatcctggtatggggaaatccagatgacccagagcccgagcagcctgagcgcgagcgtgggtgaccgtgttaccattacctgccgtgcgagccaagatgtgaacaccgcggttgcgtggtatcagcaaaagccgggcaaagcgccgaagctgctgatctacagcgcgagcttcctgtatagcggtgtgccgagccgttttagcggcagccgtagcggcaccgacttcaccctgaccattagcagcctgcagccggaggattttgcgacctactattgccagcaacactataccaccccgccgacctttggtcaaggcaccaaagttgaaatcaagagcgcggccgcactcgagc